European Patent Application EP 4 803 618 A1, published September 9, 2026. Title: A novel serine hydroxymethyltransferase variant and a method for producing purine nucleotides or glycine using the same. Applicant: CJ CheilJedang Corporation. Application KR. The sequence listing filed with the application follows.

SEQUENCE LISTING (51 sequences)

SEQ ID NO: 1 - DNA, 44 bp, synthetic construct
  source 1..44: mol_type = other DNA
cccaacgaaaggaaacactccatatgactacccagaattcttcc

SEQ ID NO: 2 - DNA, 48 bp, synthetic construct
  source 1..48: mol_type = other DNA
actggcggccgttactagtgggatccttagacgatcttccagtcttcc

SEQ ID NO: 3 - DNA, 45 bp, synthetic construct
  source 1..45: mol_type = other DNA
caagcttggtaccgagctcgcatcaccacgagttccttcaggcta

SEQ ID NO: 4 - DNA, 47 bp, synthetic construct
  source 1..47: mol_type = other DNA
gaagaattctgggtagtcatatggagtgtttcctttcgttgggtacg

SEQ ID NO: 5 - DNA, 20 bp, synthetic construct
  source 1..20: mol_type = other DNA
gaatactgtgaacttgctgg

SEQ ID NO: 6 - DNA, 20 bp, synthetic construct
  source 1..20: mol_type = other DNA
ttccgctagggacttctcca

SEQ ID NO: 7 - DNA, 38 bp, synthetic construct
  source 1..38: mol_type = other DNA
aattcgagctcggtacccactacggtggatgtgagcac

SEQ ID NO: 8 - DNA, 35 bp, synthetic construct
  source 1..35: mol_type = other DNA
ggtgcatgcttctgcatccaggccgcgggtagcca

SEQ ID NO: 9 - DNA, 35 bp, synthetic construct
  source 1..35: mol_type = other DNA
ctggatgcagaagcatgcaccgaggtggcagacat

SEQ ID NO: 10 - DNA, 38 bp, synthetic construct
  source 1..38: mol_type = other DNA
cgactctagaggatcccccgtcagcatcgatggtttcc

SEQ ID NO: 11 - DNA, 35 bp, synthetic construct
  source 1..35: mol_type = other DNA
gcgtgcgcgcagcctctgggtatcggcgttcttgc

SEQ ID NO: 12 - DNA, 35 bp, synthetic construct
  source 1..35: mol_type = other DNA
cgccgatacccagaggctgcgcgcacgcgtggaca

SEQ ID NO: 13 - DNA, 35 bp, synthetic construct
  source 1..35: mol_type = other DNA
aagcttgtccacgcgtacgcgcagcttctgggtat

SEQ ID NO: 14 - DNA, 35 bp, synthetic construct
  source 1..35: mol_type = other DNA
aagctgcgcgtacgcgtggacaagcttgctgagca

SEQ ID NO: 15 - DNA, 35 bp, synthetic construct
  source 1..35: mol_type = other DNA
tgtccacgcgtacgcgcagcctctgggtatcggcg

SEQ ID NO: 16 - DNA, 35 bp, synthetic construct
  source 1..35: mol_type = other DNA
cagaggctgcgcgtacgcgtggacaagcttgctga

SEQ ID NO: 17 - DNA, 20 bp, synthetic construct
  source 1..20: mol_type = other DNA
gcggacctgcgcaattctga

SEQ ID NO: 18 - DNA, 20 bp, synthetic construct
  source 1..20: mol_type = other DNA
cagaggatgcggataagcag

SEQ ID NO: 19 - DNA, 39 bp, synthetic construct
  source 1..39: mol_type = other DNA
aattcgagctcggtacccgatgatcgcgtctgagaactt

SEQ ID NO: 20 - DNA, 30 bp, synthetic construct
  source 1..30: mol_type = other DNA
tgcaacctcagtgcatgcaggaatatcgaa

SEQ ID NO: 21 - DNA, 30 bp, synthetic construct
  source 1..30: mol_type = other DNA
ttcgatattcctgcatgcactgaggttgca

SEQ ID NO: 22 - DNA, 39 bp, synthetic construct
  source 1..39: mol_type = other DNA
cgactctagaggatccccctttaagctcataaccaacgt

SEQ ID NO: 23 - DNA, 33 bp, synthetic construct
  source 1..33: mol_type = other DNA
tacacggccacgcagacgctcaatgtctgcgga

SEQ ID NO: 24 - DNA, 33 bp, synthetic construct
  source 1..33: mol_type = other DNA
tccgcagacattgagcgtctgcgtggccgtgta

SEQ ID NO: 25 - DNA, 31 bp, synthetic construct
  source 1..31: mol_type = other DNA
agctttgctacacggacacgcagagactcaa

SEQ ID NO: 26 - DNA, 31 bp, synthetic construct
  source 1..31: mol_type = other DNA
ttgagtctctgcgtgtccgtgtagcaaagct

SEQ ID NO: 27 - DNA, 37 bp, synthetic construct
  source 1..37: mol_type = other DNA
gctttgctacacggacacgcagacgctcaatgtctgc

SEQ ID NO: 28 - DNA, 37 bp, synthetic construct
  source 1..37: mol_type = other DNA
gcagacattgagcgtctgcgtgtccgtgtagcaaagc

SEQ ID NO: 29 - DNA, 18 bp, synthetic construct
  source 1..18: mol_type = other DNA
cccaggtcagcagggtgg

SEQ ID NO: 30 - DNA, 18 bp, synthetic construct
  source 1..18: mol_type = other DNA
ctcaatgacgcctgcaca

SEQ ID NO: 31 - protein, 433 aa, Corynebacterium stationis
MTTQNSSDAQYQEMRDLDPEVYAAINGEIARQRDTLEMIASENFVPRAVLQAQGSVLTNKYAEGYPGRRYYGGCEHVDIVEDLARDRAKALFGAEFANVQPHSGAQANAAVLASLINPGDKILGLSLAHGGHLTHGMKLNFSGKLYEVAAYEVDAETNRIDMDKLREQAIAEKPQVIIAGWSAYPRTLDFEAYRSIADEVGAYLWTDMAHFAGLVAADLYPNPVPHSDIVSTTVHKTLGGPRSGMILAKQDYAKKLNSAVFPGQQGGPLMHVVAAKAIAMKVAASEEFRDRQVRTLEGAKILAERLTTPEAKAAGVDVLTGGTDVHLVLADLRNSEMDGQQAEDLLHEVGITVNRNAVPNDPRPPMVTSGLRIGTSALATRGLDAEAFTEVADIIGTALTDGKNADTQKLRARVDKLAEQFPLYEGLEDWKIV

SEQ ID NO: 32 - protein, 433 aa, synthetic construct
MTTQNSSDAQYQEMRDLDPEVYAAINGEIARQRDTLEMIASENFVPRAVLQAQGSVLTNKYAEGYPGRRYYGGCEHVDIVEDLARDRAKALFGAEFANVQPHSGAQANAAVLASLINPGDKILGLSLAHGGHLTHGMKLNFSGKLYEVAAYEVDAETNRIDMDKLREQAIAEKPQVIIAGWSAYPRTLDFEAYRSIADEVGAYLWTDMAHFAGLVAADLYPNPVPHSDIVSTTVHKTLGGPRSGMILAKQDYAKKLNSAVFPGQQGGPLMHVVAAKAIAMKVAASEEFRDRQVRTLEGAKILAERLTTPEAKAAGVDVLTGGTDVHLVLADLRNSEMDGQQAEDLLHEVGITVNRNAVPNDPRPPMVTSGLRIGTSALATRGLDAEACTEVADIIGTALTDGKNADTQKLRARVDKLAEQFPLYEGLEDWKIV

SEQ ID NO: 33 - protein, 433 aa, synthetic construct
MTTQNSSDAQYQEMRDLDPEVYAAINGEIARQRDTLEMIASENFVPRAVLQAQGSVLTNKYAEGYPGRRYYGGCEHVDIVEDLARDRAKALFGAEFANVQPHSGAQANAAVLASLINPGDKILGLSLAHGGHLTHGMKLNFSGKLYEVAAYEVDAETNRIDMDKLREQAIAEKPQVIIAGWSAYPRTLDFEAYRSIADEVGAYLWTDMAHFAGLVAADLYPNPVPHSDIVSTTVHKTLGGPRSGMILAKQDYAKKLNSAVFPGQQGGPLMHVVAAKAIAMKVAASEEFRDRQVRTLEGAKILAERLTTPEAKAAGVDVLTGGTDVHLVLADLRNSEMDGQQAEDLLHEVGITVNRNAVPNDPRPPMVTSGLRIGTSALATRGLDAEAFTEVADIIGTALTDGKNADTQRLRARVDKLAEQFPLYEGLEDWKIV

SEQ ID NO: 34 - protein, 433 aa, synthetic construct
MTTQNSSDAQYQEMRDLDPEVYAAINGEIARQRDTLEMIASENFVPRAVLQAQGSVLTNKYAEGYPGRRYYGGCEHVDIVEDLARDRAKALFGAEFANVQPHSGAQANAAVLASLINPGDKILGLSLAHGGHLTHGMKLNFSGKLYEVAAYEVDAETNRIDMDKLREQAIAEKPQVIIAGWSAYPRTLDFEAYRSIADEVGAYLWTDMAHFAGLVAADLYPNPVPHSDIVSTTVHKTLGGPRSGMILAKQDYAKKLNSAVFPGQQGGPLMHVVAAKAIAMKVAASEEFRDRQVRTLEGAKILAERLTTPEAKAAGVDVLTGGTDVHLVLADLRNSEMDGQQAEDLLHEVGITVNRNAVPNDPRPPMVTSGLRIGTSALATRGLDAEAFTEVADIIGTALTDGKNADTQKLRVRVDKLAEQFPLYEGLEDWKIV

SEQ ID NO: 35 - protein, 433 aa, synthetic construct
MTTQNSSDAQYQEMRDLDPEVYAAINGEIARQRDTLEMIASENFVPRAVLQAQGSVLTNKYAEGYPGRRYYGGCEHVDIVEDLARDRAKALFGAEFANVQPHSGAQANAAVLASLINPGDKILGLSLAHGGHLTHGMKLNFSGKLYEVAAYEVDAETNRIDMDKLREQAIAEKPQVIIAGWSAYPRTLDFEAYRSIADEVGAYLWTDMAHFAGLVAADLYPNPVPHSDIVSTTVHKTLGGPRSGMILAKQDYAKKLNSAVFPGQQGGPLMHVVAAKAIAMKVAASEEFRDRQVRTLEGAKILAERLTTPEAKAAGVDVLTGGTDVHLVLADLRNSEMDGQQAEDLLHEVGITVNRNAVPNDPRPPMVTSGLRIGTSALATRGLDAEACTEVADIIGTALTDGKNADTQRLRVRVDKLAEQFPLYEGLEDWKIV

SEQ ID NO: 36 - DNA, 1302 bp, Corynebacterium stationis
  source 1..1302: mol_type = other DNA
atgactacccagaattcttccgatgctcagtaccaggaaatgcgtgacttagacccagaggtctatgcagcaattaacggtgaaattgctcgtcagcgcgataccctggagatgattgcgtcggagaactttgttcctcgtgcagtcttgcaggcacagggttccgtccttaccaacaagtacgcagagggctacccaggtcgccgctactacggtggatgtgagcacgtcgatatcgtcgaagatctggcgcgtgaccgcgctaaggctctgttcggcgctgagtttgccaatgtacagccacactccggtgcacaggcaaacgctgccgtccttgcttctcttatcaacccaggcgataagatcttgggcctttctttggctcacggtggtcacctgacccacggcatgaagctgaacttctccggcaagctctacgaagtagctgcctacgaagtcgatgcagaaaccaaccgtatcgacatggacaagctgcgtgagcaggctattgcagaaaagccacaggtcatcatcgctggctggtctgcatacccacgcactctggattttgaagcataccgttccatcgcggatgaagtgggggcttacctgtggaccgatatggcacactttgctggtctcgttgccgctgatctgtacccaaatccagttccacactctgacattgtttccaccaccgtgcacaagaccctgggcggtcctcgctccggcatgatcctggctaagcaggactacgctaagaagctcaactctgcagtcttcccaggccagcagggtggccctttgatgcatgtggttgcagcgaaggcaattgccatgaaggttgctgcttccgaagaattccgtgaccgtcaggtccgtactctggaaggcgcgaagattcttgctgagcgcttgaccactcctgaggcaaaggcagcaggcgttgacgttctcactggcggcaccgacgtgcacttggttcttgcggacctgcgcaattctgagatggatggccagcaggcagaagacctcctgcacgaggtcggcatcaccgttaaccgcaacgcggttccaaacgatccacgtccaccaatggtgacctctggtctgcgtatcggtacttccgctctggctacccgcggcctggatgcagaagcattcaccgaggtggcagacatcatcggcaccgcgcttaccgatggcaagaacgccgatacccagaagctgcgcgcacgcgtggacaagcttgctgagcagttcccactctacgagggcttggaagactggaagatcgtctaa

SEQ ID NO: 37 - DNA, 1302 bp, synthetic construct
  source 1..1302: mol_type = other DNA
atgactacccagaattcttccgatgctcagtaccaggaaatgcgtgacttagacccagaggtctatgcagcaattaacggtgaaattgctcgtcagcgcgataccctggagatgattgcgtcggagaactttgttcctcgtgcagtcttgcaggcacagggttccgtccttaccaacaagtacgcagagggctacccaggtcgccgctactacggtggatgtgagcacgtcgatatcgtcgaagatctggcgcgtgaccgcgctaaggctctgttcggcgctgagtttgccaatgtacagccacactccggtgcacaggcaaacgctgccgtccttgcttctcttatcaacccaggcgataagatcttgggcctttctttggctcacggtggtcacctgacccacggcatgaagctgaacttctccggcaagctctacgaagtagctgcctacgaagtcgatgcagaaaccaaccgtatcgacatggacaagctgcgtgagcaggctattgcagaaaagccacaggtcatcatcgctggctggtctgcatacccacgcactctggattttgaagcataccgttccatcgcggatgaagtgggggcttacctgtggaccgatatggcacactttgctggtctcgttgccgctgatctgtacccaaatccagttccacactctgacattgtttccaccaccgtgcacaagaccctgggcggtcctcgctccggcatgatcctggctaagcaggactacgctaagaagctcaactctgcagtcttcccaggccagcagggtggccctttgatgcatgtggttgcagcgaaggcaattgccatgaaggttgctgcttccgaagaattccgtgaccgtcaggtccgtactctggaaggcgcgaagattcttgctgagcgcttgaccactcctgaggcaaaggcagcaggcgttgacgttctcactggcggcaccgacgtgcacttggttcttgcggacctgcgcaattctgagatggatggccagcaggcagaagacctcctgcacgaggtcggcatcaccgttaaccgcaacgcggttccaaacgatccacgtccaccaatggtgacctctggtctgcgtatcggtacttccgctctggctacccgcggcctggatgcagaagcatgcaccgaggtggcagacatcatcggcaccgcgcttaccgatggcaagaacgccgatacccagaagctgcgcgcacgcgtggacaagcttgctgagcagttcccactctacgagggcttggaagactggaagatcgtctaa

SEQ ID NO: 38 - DNA, 1302 bp, synthetic construct
  source 1..1302: mol_type = other DNA
atgactacccagaattcttccgatgctcagtaccaggaaatgcgtgacttagacccagaggtctatgcagcaattaacggtgaaattgctcgtcagcgcgataccctggagatgattgcgtcggagaactttgttcctcgtgcagtcttgcaggcacagggttccgtccttaccaacaagtacgcagagggctacccaggtcgccgctactacggtggatgtgagcacgtcgatatcgtcgaagatctggcgcgtgaccgcgctaaggctctgttcggcgctgagtttgccaatgtacagccacactccggtgcacaggcaaacgctgccgtccttgcttctcttatcaacccaggcgataagatcttgggcctttctttggctcacggtggtcacctgacccacggcatgaagctgaacttctccggcaagctctacgaagtagctgcctacgaagtcgatgcagaaaccaaccgtatcgacatggacaagctgcgtgagcaggctattgcagaaaagccacaggtcatcatcgctggctggtctgcatacccacgcactctggattttgaagcataccgttccatcgcggatgaagtgggggcttacctgtggaccgatatggcacactttgctggtctcgttgccgctgatctgtacccaaatccagttccacactctgacattgtttccaccaccgtgcacaagaccctgggcggtcctcgctccggcatgatcctggctaagcaggactacgctaagaagctcaactctgcagtcttcccaggccagcagggtggccctttgatgcatgtggttgcagcgaaggcaattgccatgaaggttgctgcttccgaagaattccgtgaccgtcaggtccgtactctggaaggcgcgaagattcttgctgagcgcttgaccactcctgaggcaaaggcagcaggcgttgacgttctcactggcggcaccgacgtgcacttggttcttgcggacctgcgcaattctgagatggatggccagcaggcagaagacctcctgcacgaggtcggcatcaccgttaaccgcaacgcggttccaaacgatccacgtccaccaatggtgacctctggtctgcgtatcggtacttccgctctggctacccgcggcctggatgcagaagcattcaccgaggtggcagacatcatcggcaccgcgcttaccgatggcaagaacgccgatacccagaggctgcgcgcacgcgtggacaagcttgctgagcagttcccactctacgagggcttggaagactggaagatcgtctaa

SEQ ID NO: 39 - DNA, 1302 bp, synthetic construct
  source 1..1302: mol_type = other DNA
atgactacccagaattcttccgatgctcagtaccaggaaatgcgtgacttagacccagaggtctatgcagcaattaacggtgaaattgctcgtcagcgcgataccctggagatgattgcgtcggagaactttgttcctcgtgcagtcttgcaggcacagggttccgtccttaccaacaagtacgcagagggctacccaggtcgccgctactacggtggatgtgagcacgtcgatatcgtcgaagatctggcgcgtgaccgcgctaaggctctgttcggcgctgagtttgccaatgtacagccacactccggtgcacaggcaaacgctgccgtccttgcttctcttatcaacccaggcgataagatcttgggcctttctttggctcacggtggtcacctgacccacggcatgaagctgaacttctccggcaagctctacgaagtagctgcctacgaagtcgatgcagaaaccaaccgtatcgacatggacaagctgcgtgagcaggctattgcagaaaagccacaggtcatcatcgctggctggtctgcatacccacgcactctggattttgaagcataccgttccatcgcggatgaagtgggggcttacctgtggaccgatatggcacactttgctggtctcgttgccgctgatctgtacccaaatccagttccacactctgacattgtttccaccaccgtgcacaagaccctgggcggtcctcgctccggcatgatcctggctaagcaggactacgctaagaagctcaactctgcagtcttcccaggccagcagggtggccctttgatgcatgtggttgcagcgaaggcaattgccatgaaggttgctgcttccgaagaattccgtgaccgtcaggtccgtactctggaaggcgcgaagattcttgctgagcgcttgaccactcctgaggcaaaggcagcaggcgttgacgttctcactggcggcaccgacgtgcacttggttcttgcggacctgcgcaattctgagatggatggccagcaggcagaagacctcctgcacgaggtcggcatcaccgttaaccgcaacgcggttccaaacgatccacgtccaccaatggtgacctctggtctgcgtatcggtacttccgctctggctacccgcggcctggatgcagaagcattcaccgaggtggcagacatcatcggcaccgcgcttaccgatggcaagaacgccgatacccagaagctgcgcgtacgcgtggacaagcttgctgagcagttcccactctacgagggcttggaagactggaagatcgtctaa

SEQ ID NO: 40 - DNA, 1302 bp, synthetic construct
  source 1..1302: mol_type = other DNA
atgactacccagaattcttccgatgctcagtaccaggaaatgcgtgacttagacccagaggtctatgcagcaattaacggtgaaattgctcgtcagcgcgataccctggagatgattgcgtcggagaactttgttcctcgtgcagtcttgcaggcacagggttccgtccttaccaacaagtacgcagagggctacccaggtcgccgctactacggtggatgtgagcacgtcgatatcgtcgaagatctggcgcgtgaccgcgctaaggctctgttcggcgctgagtttgccaatgtacagccacactccggtgcacaggcaaacgctgccgtccttgcttctcttatcaacccaggcgataagatcttgggcctttctttggctcacggtggtcacctgacccacggcatgaagctgaacttctccggcaagctctacgaagtagctgcctacgaagtcgatgcagaaaccaaccgtatcgacatggacaagctgcgtgagcaggctattgcagaaaagccacaggtcatcatcgctggctggtctgcatacccacgcactctggattttgaagcataccgttccatcgcggatgaagtgggggcttacctgtggaccgatatggcacactttgctggtctcgttgccgctgatctgtacccaaatccagttccacactctgacattgtttccaccaccgtgcacaagaccctgggcggtcctcgctccggcatgatcctggctaagcaggactacgctaagaagctcaactctgcagtcttcccaggccagcagggtggccctttgatgcatgtggttgcagcgaaggcaattgccatgaaggttgctgcttccgaagaattccgtgaccgtcaggtccgtactctggaaggcgcgaagattcttgctgagcgcttgaccactcctgaggcaaaggcagcaggcgttgacgttctcactggcggcaccgacgtgcacttggttcttgcggacctgcgcaattctgagatggatggccagcaggcagaagacctcctgcacgaggtcggcatcaccgttaaccgcaacgcggttccaaacgatccacgtccaccaatggtgacctctggtctgcgtatcggtacttccgctctggctacccgcggcctggatgcagaagcatgcaccgaggtggcagacatcatcggcaccgcgcttaccgatggcaagaacgccgatacccagaggctgcgcgtacgcgtggacaagcttgctgagcagttcccactctacgagggcttggaagactggaagatcgtctaa

SEQ ID NO: 41 - protein, 434 aa, Corynebacterium glutamicum
MTDAHQADDVRYQPLNELDPEVAAAIAGELARQRDTLEMIASENFVPRSVLQAQGSVLTNKYAEGYPGRRYYGGCEQVDIIEDLARDRAKALFGAEFANVQPHSGAQANAAVLMTLAEPGDKIMGLSLAHGGHLTHGMKLNFSGKLYEVVAYGVDPETMRVDMDQVREIALKEQPKVIIAGWSAYPRHLDFEAFQSIAAEVGAKLWVDMAHFAGLVAAGLHPSPVPYSDVVSSTVHKTLGGPRSGIILAKQEYAKKLNSSVFPGQQGGPLMHAVAAKATSLKIAGTEQFRDRQARTLEGARILAERLTASDAKAAGVDVLTGGTDVHLVLADLRNSQMDGQQAEDLLHEVGITVNRNAVPFDPRPPMVTSGLRIGTPALATRGFDIPAFTEVADIIGTALANGKSADIESLRGRVAKLAADYPLYEGLEDWTIV

SEQ ID NO: 42 - protein, 434 aa, synthetic construct
MTDAHQADDVRYQPLNELDPEVAAAIAGELARQRDTLEMIASENFVPRSVLQAQGSVLTNKYAEGYPGRRYYGGCEQVDIIEDLARDRAKALFGAEFANVQPHSGAQANAAVLMTLAEPGDKIMGLSLAHGGHLTHGMKLNFSGKLYEVVAYGVDPETMRVDMDQVREIALKEQPKVIIAGWSAYPRHLDFEAFQSIAAEVGAKLWVDMAHFAGLVAAGLHPSPVPYSDVVSSTVHKTLGGPRSGIILAKQEYAKKLNSSVFPGQQGGPLMHAVAAKATSLKIAGTEQFRDRQARTLEGARILAERLTASDAKAAGVDVLTGGTDVHLVLADLRNSQMDGQQAEDLLHEVGITVNRNAVPFDPRPPMVTSGLRIGTPALATRGFDIPACTEVADIIGTALANGKSADIESLRGRVAKLAADYPLYEGLEDWTIV

SEQ ID NO: 43 - protein, 434 aa, synthetic construct
MTDAHQADDVRYQPLNELDPEVAAAIAGELARQRDTLEMIASENFVPRSVLQAQGSVLTNKYAEGYPGRRYYGGCEQVDIIEDLARDRAKALFGAEFANVQPHSGAQANAAVLMTLAEPGDKIMGLSLAHGGHLTHGMKLNFSGKLYEVVAYGVDPETMRVDMDQVREIALKEQPKVIIAGWSAYPRHLDFEAFQSIAAEVGAKLWVDMAHFAGLVAAGLHPSPVPYSDVVSSTVHKTLGGPRSGIILAKQEYAKKLNSSVFPGQQGGPLMHAVAAKATSLKIAGTEQFRDRQARTLEGARILAERLTASDAKAAGVDVLTGGTDVHLVLADLRNSQMDGQQAEDLLHEVGITVNRNAVPFDPRPPMVTSGLRIGTPALATRGFDIPAFTEVADIIGTALANGKSADIERLRGRVAKLAADYPLYEGLEDWTIV

SEQ ID NO: 44 - protein, 434 aa, synthetic construct
MTDAHQADDVRYQPLNELDPEVAAAIAGELARQRDTLEMIASENFVPRSVLQAQGSVLTNKYAEGYPGRRYYGGCEQVDIIEDLARDRAKALFGAEFANVQPHSGAQANAAVLMTLAEPGDKIMGLSLAHGGHLTHGMKLNFSGKLYEVVAYGVDPETMRVDMDQVREIALKEQPKVIIAGWSAYPRHLDFEAFQSIAAEVGAKLWVDMAHFAGLVAAGLHPSPVPYSDVVSSTVHKTLGGPRSGIILAKQEYAKKLNSSVFPGQQGGPLMHAVAAKATSLKIAGTEQFRDRQARTLEGARILAERLTASDAKAAGVDVLTGGTDVHLVLADLRNSQMDGQQAEDLLHEVGITVNRNAVPFDPRPPMVTSGLRIGTPALATRGFDIPAFTEVADIIGTALANGKSADIESLRVRVAKLAADYPLYEGLEDWTIV

SEQ ID NO: 45 - protein, 434 aa, synthetic construct
MTDAHQADDVRYQPLNELDPEVAAAIAGELARQRDTLEMIASENFVPRSVLQAQGSVLTNKYAEGYPGRRYYGGCEQVDIIEDLARDRAKALFGAEFANVQPHSGAQANAAVLMTLAEPGDKIMGLSLAHGGHLTHGMKLNFSGKLYEVVAYGVDPETMRVDMDQVREIALKEQPKVIIAGWSAYPRHLDFEAFQSIAAEVGAKLWVDMAHFAGLVAAGLHPSPVPYSDVVSSTVHKTLGGPRSGIILAKQEYAKKLNSSVFPGQQGGPLMHAVAAKATSLKIAGTEQFRDRQARTLEGARILAERLTASDAKAAGVDVLTGGTDVHLVLADLRNSQMDGQQAEDLLHEVGITVNRNAVPFDPRPPMVTSGLRIGTPALATRGFDIPACTEVADIIGTALANGKSADIERLRVRVAKLAADYPLYEGLEDWTIV

SEQ ID NO: 46 - DNA, 1305 bp, Corynebacterium glutamicum
  source 1..1305: mol_type = other DNA
atgaccgatgcccaccaagcggacgatgtccgttaccagccactgaacgagcttgatcctgaggtggctgctgccatcgctggggaacttgcccgtcaacgcgatacattagagatgatcgcgtctgagaacttcgttccccgttctgttttgcaggcgcagggttctgttcttaccaataagtatgccgagggttaccctggccgccgttactacggtggttgcgaacaagttgacatcattgaggatcttgcacgtgatcgtgcgaaggctctcttcggtgcagagttcgccaatgttcagcctcactctggcgcacaggctaatgctgctgtgctgatgactttggctgagccaggcgacaagatcatgggtctgtctttggctcatggtggtcacttgacccacggaatgaagttgaacttctccggaaagctgtacgaggttgttgcgtacggtgttgatcctgagaccatgcgtgttgatatggatcaggttcgtgagattgctctgaaggagcagccaaaggtaattatcgctggctggtctgcataccctcgccaccttgatttcgaggctttccagtctattgctgcggaagttggcgcgaagctgtgggtcgatatggctcacttcgctggtcttgttgctgctggtttgcacccaagcccagttccttactctgatgttgtttcttccactgtccacaagactttgggtggacctcgttccggcatcattctggctaagcaggagtacgcgaagaagctgaactcttccgtattcccaggtcagcagggtggtcctttgatgcacgcagttgctgcgaaggctacttctttgaagattgctggcactgagcagttccgtgaccgtcaggctcgcacgttggagggtgctcgcattcttgctgagcgtctgactgcttctgatgcgaaggccgctggcgtggatgtcttgaccggtggcactgatgtgcacttggttttggctgatctgcgtaactcccagatggatggccagcaggcggaagatctgctgcacgaggttggtatcactgtgaaccgtaacgcggttcctttcgatcctcgtccaccaatggttacttctggtctgcgtattggtactcctgcgctggctacccgtggtttcgatattcctgcattcactgaggttgcagacatcattggtactgctttggctaatggtaagtccgcagacattgagtctctgcgtggccgtgtagcaaagcttgctgcagattacccactgtatgagggcttggaagactggaccatcgtctaa

SEQ ID NO: 47 - DNA, 1305 bp, synthetic construct
  source 1..1305: mol_type = other DNA
atgaccgatgcccaccaagcggacgatgtccgttaccagccactgaacgagcttgatcctgaggtggctgctgccatcgctggggaacttgcccgtcaacgcgatacattagagatgatcgcgtctgagaacttcgttccccgttctgttttgcaggcgcagggttctgttcttaccaataagtatgccgagggttaccctggccgccgttactacggtggttgcgaacaagttgacatcattgaggatcttgcacgtgatcgtgcgaaggctctcttcggtgcagagttcgccaatgttcagcctcactctggcgcacaggctaatgctgctgtgctgatgactttggctgagccaggcgacaagatcatgggtctgtctttggctcatggtggtcacttgacccacggaatgaagttgaacttctccggaaagctgtacgaggttgttgcgtacggtgttgatcctgagaccatgcgtgttgatatggatcaggttcgtgagattgctctgaaggagcagccaaaggtaattatcgctggctggtctgcataccctcgccaccttgatttcgaggctttccagtctattgctgcggaagttggcgcgaagctgtgggtcgatatggctcacttcgctggtcttgttgctgctggtttgcacccaagcccagttccttactctgatgttgtttcttccactgtccacaagactttgggtggacctcgttccggcatcattctggctaagcaggagtacgcgaagaagctgaactcttccgtattcccaggtcagcagggtggtcctttgatgcacgcagttgctgcgaaggctacttctttgaagattgctggcactgagcagttccgtgaccgtcaggctcgcacgttggagggtgctcgcattcttgctgagcgtctgactgcttctgatgcgaaggccgctggcgtggatgtcttgaccggtggcactgatgtgcacttggttttggctgatctgcgtaactcccagatggatggccagcaggcggaagatctgctgcacgaggttggtatcactgtgaaccgtaacgcggttcctttcgatcctcgtccaccaatggttacttctggtctgcgtattggtactcctgcgctggctacccgtggtttcgatattcctgcatgcactgaggttgcagacatcattggtactgctttggctaatggtaagtccgcagacattgagtctctgcgtggccgtgtagcaaagcttgctgcagattacccactgtatgagggcttggaagactggaccatcgtctaa

SEQ ID NO: 48 - DNA, 1305 bp, synthetic construct
  source 1..1305: mol_type = other DNA
atgaccgatgcccaccaagcggacgatgtccgttaccagccactgaacgagcttgatcctgaggtggctgctgccatcgctggggaacttgcccgtcaacgcgatacattagagatgatcgcgtctgagaacttcgttccccgttctgttttgcaggcgcagggttctgttcttaccaataagtatgccgagggttaccctggccgccgttactacggtggttgcgaacaagttgacatcattgaggatcttgcacgtgatcgtgcgaaggctctcttcggtgcagagttcgccaatgttcagcctcactctggcgcacaggctaatgctgctgtgctgatgactttggctgagccaggcgacaagatcatgggtctgtctttggctcatggtggtcacttgacccacggaatgaagttgaacttctccggaaagctgtacgaggttgttgcgtacggtgttgatcctgagaccatgcgtgttgatatggatcaggttcgtgagattgctctgaaggagcagccaaaggtaattatcgctggctggtctgcataccctcgccaccttgatttcgaggctttccagtctattgctgcggaagttggcgcgaagctgtgggtcgatatggctcacttcgctggtcttgttgctgctggtttgcacccaagcccagttccttactctgatgttgtttcttccactgtccacaagactttgggtggacctcgttccggcatcattctggctaagcaggagtacgcgaagaagctgaactcttccgtattcccaggtcagcagggtggtcctttgatgcacgcagttgctgcgaaggctacttctttgaagattgctggcactgagcagttccgtgaccgtcaggctcgcacgttggagggtgctcgcattcttgctgagcgtctgactgcttctgatgcgaaggccgctggcgtggatgtcttgaccggtggcactgatgtgcacttggttttggctgatctgcgtaactcccagatggatggccagcaggcggaagatctgctgcacgaggttggtatcactgtgaaccgtaacgcggttcctttcgatcctcgtccaccaatggttacttctggtctgcgtattggtactcctgcgctggctacccgtggtttcgatattcctgcattcactgaggttgcagacatcattggtactgctttggctaatggtaagtccgcagacattgagcgtctgcgtggccgtgtagcaaagcttgctgcagattacccactgtatgagggcttggaagactggaccatcgtctaa

SEQ ID NO: 49 - DNA, 1305 bp, synthetic construct
  source 1..1305: mol_type = other DNA
atgaccgatgcccaccaagcggacgatgtccgttaccagccactgaacgagcttgatcctgaggtggctgctgccatcgctggggaacttgcccgtcaacgcgatacattagagatgatcgcgtctgagaacttcgttccccgttctgttttgcaggcgcagggttctgttcttaccaataagtatgccgagggttaccctggccgccgttactacggtggttgcgaacaagttgacatcattgaggatcttgcacgtgatcgtgcgaaggctctcttcggtgcagagttcgccaatgttcagcctcactctggcgcacaggctaatgctgctgtgctgatgactttggctgagccaggcgacaagatcatgggtctgtctttggctcatggtggtcacttgacccacggaatgaagttgaacttctccggaaagctgtacgaggttgttgcgtacggtgttgatcctgagaccatgcgtgttgatatggatcaggttcgtgagattgctctgaaggagcagccaaaggtaattatcgctggctggtctgcataccctcgccaccttgatttcgaggctttccagtctattgctgcggaagttggcgcgaagctgtgggtcgatatggctcacttcgctggtcttgttgctgctggtttgcacccaagcccagttccttactctgatgttgtttcttccactgtccacaagactttgggtggacctcgttccggcatcattctggctaagcaggagtacgcgaagaagctgaactcttccgtattcccaggtcagcagggtggtcctttgatgcacgcagttgctgcgaaggctacttctttgaagattgctggcactgagcagttccgtgaccgtcaggctcgcacgttggagggtgctcgcattcttgctgagcgtctgactgcttctgatgcgaaggccgctggcgtggatgtcttgaccggtggcactgatgtgcacttggttttggctgatctgcgtaactcccagatggatggccagcaggcggaagatctgctgcacgaggttggtatcactgtgaaccgtaacgcggttcctttcgatcctcgtccaccaatggttacttctggtctgcgtattggtactcctgcgctggctacccgtggtttcgatattcctgcattcactgaggttgcagacatcattggtactgctttggctaatggtaagtccgcagacattgagtctctgcgtgtccgtgtagcaaagcttgctgcagattacccactgtatgagggcttggaagactggaccatcgtctaa

SEQ ID NO: 50 - DNA, 1305 bp, synthetic construct
  source 1..1305: mol_type = other DNA
atgaccgatgcccaccaagcggacgatgtccgttaccagccactgaacgagcttgatcctgaggtggctgctgccatcgctggggaacttgcccgtcaacgcgatacattagagatgatcgcgtctgagaacttcgttccccgttctgttttgcaggcgcagggttctgttcttaccaataagtatgccgagggttaccctggccgccgttactacggtggttgcgaacaagttgacatcattgaggatcttgcacgtgatcgtgcgaaggctctcttcggtgcagagttcgccaatgttcagcctcactctggcgcacaggctaatgctgctgtgctgatgactttggctgagccaggcgacaagatcatgggtctgtctttggctcatggtggtcacttgacccacggaatgaagttgaacttctccggaaagctgtacgaggttgttgcgtacggtgttgatcctgagaccatgcgtgttgatatggatcaggttcgtgagattgctctgaaggagcagccaaaggtaattatcgctggctggtctgcataccctcgccaccttgatttcgaggctttccagtctattgctgcggaagttggcgcgaagctgtgggtcgatatggctcacttcgctggtcttgttgctgctggtttgcacccaagcccagttccttactctgatgttgtttcttccactgtccacaagactttgggtggacctcgttccggcatcattctggctaagcaggagtacgcgaagaagctgaactcttccgtattcccaggtcagcagggtggtcctttgatgcacgcagttgctgcgaaggctacttctttgaagattgctggcactgagcagttccgtgaccgtcaggctcgcacgttggagggtgctcgcattcttgctgagcgtctgactgcttctgatgcgaaggccgctggcgtggatgtcttgaccggtggcactgatgtgcacttggttttggctgatctgcgtaactcccagatggatggccagcaggcggaagatctgctgcacgaggttggtatcactgtgaaccgtaacgcggttcctttcgatcctcgtccaccaatggttacttctggtctgcgtattggtactcctgcgctggctacccgtggtttcgatattcctgcatgcactgaggttgcagacatcattggtactgctttggctaatggtaagtccgcagacattgagcgtctgcgtgtccgtgtagcaaagcttgctgcagattacccactgtatgagggcttggaagactggaccatcgtctaa

SEQ ID NO: 51 - DNA, 5802 bp, synthetic construct
  source 1..5802: mol_type = other DNA
gttcgcttgctgtccataaaaccgcccagtctagctatcgccatgtaagcccactgcaagctacctgctttctctttgcgcttgcgttttcccttgtccagatagcccagtagctgacattcatccggggtcagcaccgtttctgcggactggctttctacgtgttccgcttcctttagcagcccttgcgccctgagtgcttgcggcagcgtgaagctagcttttatcgccattcgccattcaggctgcgcaactgttgggaagggcgatcggtgcgggcctcttcgctattacgccagctggcgaaagggggatgtgctgcaaggcgattaagttgggtaacgccagggttttcccagtcacgacgttgtaaaacgacggccagtgaattcgagctcggtacccggggatcctctagagtcgacctgcaggcatgcaagcttggcgtaatcatggtcatagctgtttcctgtgtgaaattgttatccgctcacaattccacacaacatacgagccggaagcataaagtgtaaagcctggggtgcctaatgagtgagctaactcacattaattgcgttgcgctcactgcccgctttccagtcgggaaacctgtcgtgccagctgcattaatgaatcggccaacgcgcggggagaggcggtttgcgtattgggcgctcttccgcttcctcgctcactgactcgctgcgctcggtcgttcggctgcggcgagcggtatcagctcactcaaaggcggtaatacggttatccacagaatcaggggataacgcaggaaagaacatgtgagcaaaaggccagcaaaaggccaggaaccgtaaaaaggccgcgttgctggcgtttttccataggctccgcccccctgacgagcatcacaaaaatcgacgctcaagtcagaggtggcgaaacccgacaggactataaagataccaggcgtttccccctggaagctccctcgtgcgctctcctgttccgaccctgccgcttaccggatacctgtccgcctttctcccttcgggaagcgtggcgctttctcaatgctcacgctgtaggtatctcagttcggtgtaggtcgttcgctccaagctgggctgtgtgcacgaaccccccgttcagcccgaccgctgcgccttatccggtaactatcgtcttgagtccaacccggtaagacacgacttatcgccactggcagcagccactggtaacaggattagcagagcgaggtatgtaggcggtgctacagagttcttgaagtggtggcctaactacggctacactagaaggacagtatttggtatctgcgctctgctgaagccagttaccttcggaaaaagagttggtagctcttgatccggcaaacaaaccaccgctggtagcggtggtttttttgtttgcaagcagcagattacgcgcagaaaaaaaggatctcaagaagatcctttgatcttttctacggggtctgacgctcagtggaacgaaaactcacgttaagggattttggtcatgagattatcaaaaaggatcttcacctagatccttttggggtgggcgaagaactccagcatgagatccccgcgctggaggatcatccagccctgatagaaacagaagccactggagcacctcaaaaacaccatcatacactaaatcagtaagttggcagcatcacccgacgcactttgcgccgaataaatacctgtgacggaagatcacttcgcagaataaataaatcctggtgtccctgttgataccgggaagccctgggccaacttttggcgaaaatgagacgttgatcggcacgtaagaggttccaactttcaccataatgaaataagatcactaccgggcgtattttttgagttatcgagattttcaggagctgatagaaacagaagccactggagcacctcaaaaacaccatcatacactaaatcagtaagttggcagcatcacccgacgcactttgcgccgaataaatacctgtgacggaagatcacttcgcagaataaataaatcctggtgtccctgttgataccgggaagccctgggccaacttttggcgaaaatgagacgttgatcggcacgtaagaggttccaactttcaccataatgaaataagatcactaccgggcgtattttttgagttatcgagattttcaggagctctttggcatcgtctctcgcctgtcccctcagttcagtaatttcctgcatttgcctgtttccagtcggtagatattccacaaaacagcagggaagcagcgcttttccgctgcataaccctgcttcggggtcattatagcgattttttcggtatatccatcctttttcgcacgatatacaggattttgccaaagggttcgtgtagactttccttggtgtatccaacggcgtcagccgggcaggataggtgaagtaggcccacccgcgagcgggtgttccttcttcactgtcccttattcgcacctggcggtgctcaacgggaatcctgctctgcgaggctggccggctaccgccggcgtaacagatgagggcaagcggatggctgatgaaaccaagccaaccaggaagggcagcccacctatcaaggtgtactgccttccagacgaacgaagagcgattgaggaaaaggcggcggcggccggcatgagcctgtcggcctacctgctggccgtcggccagggctacaaaatcacgggcgtcgtggactatgagcacgtccgcgagggcgtcccggaaaacgattccgaagcccaacctttcatagaaggcggcggtggaatcgaaatctcgtgatggcaggttgggcgtcgcttggtcggtcatttcgaaaaaggttaggaatacggttagccatttgcctgcttttatatagttcatatgggattcacctttatgttgataagaaataaaagaaaatgccaataggatatcggcattttcttttgcgtttttatttgttaactgttaattgtccttgttcaaggatgctgtctttgacaacagatgttttcttgcctttgatgttcagcaggaagctcggcgcaaacgttgattgtttgtctgcgtagaatcctctgtttgtcatatagcttgtaatcacgacattgtttcctttcgcttgaggtacagcgaagtgtgagtaagtaaaggttacatcgttaggcggatcaagatccatttttaacacaaggccagttttgttcagcggcttgtatgggccagttaaagaattagaaacataaccaagcatgtaaatatcgttagacgtaatgccgtcaatcgtcatttttgatccgcgggagtcagtgaacaggtaccatttgccgttcattttaaagacgttcgcgcgttcaatttcatctgttactgtgttagatgcaatcagcggtttcatcacttttttcagtgtgtaatcatcgtttagctcaatcataccgagagcgccgtttgctaactcagccgtgcgttttttatcgctttgcagaagtttttgactttcttgacggaagaatgatgtgcttttgccatagtatgctttgttaaataaagattcttcgccttggtagccatcttcagttccagtgtttgcttcaaatactaagtatttgtggcctttatcttctacgtagtgaggatctctcagcgtatggttgtcgcctgagctgtagttgccttcatcgatgaactgctgtacattttgatacgtttttccgtcaccgtcaaagattgatttataatcctctacaccgttgatgttcaaagagctgtctgatgctgatacgttaacttgtgcagttgtcagtgtttgtttgccgtaatgtttaccggagaaatcagtgtagaataaacggatttttccgtcagatgtaaatgtggctgaacctgaccattcttgtgtttggtcttttaggatagaatcatttgcatcgaatttgtcgctgtctttaaagacgcggccagcgtttttccagctgtcaatagaagtttcgccgactttttgatagaacatgtaaatcgatgtgtcatccgcatttttaggatctccggctaatgcaaagacgatgtggtagccgtgatagtttgcgacagtgccgtcagcgttttgtaatggccagctgtcccaaacgtccaggccttttgcagaagagatatttttaattgtggacgaatcaaattcagaaacttgatatttttcatttttttgctgttcagggatttgcagcatatcatggcgtgtaatatgggaaatgccgtatgtttccttatatggcttttggttcgtttctttcgcaaacgcttgagttgcgcctcctgccagcagtgcggtagtaaaggttaatactgttgcttgttttgcaaactttttgatgttcatcgttcatgtctccttttttatgtactgtgttagcggtctgcttcttccagccctcctgtttgaagatggcaagttagttacgcacaataaaaaaagacctaaaatatgtaaggggtgacgccaaagtatacactttgccctttacacattttaggtcttgcctgctttatcagtaacaaacccgcgcgatttacttttcgacctcattctattagactctcgtttggattgcaactggtctattttcctcttttgtttgatagaaaatcataaaaggatttgcagactacgggcctaaagaactaaaaaatctatctgtttcttttcattctctgtattttttatagtttctgttgcatgggcataaagttgcctttttaatcacaattcagaaaatatcataatatctcatttcactaaataatagtgaacggcaggtatatgtgatgggttaaaaaggatcaccccagagtcccgctcagaagaactcgtcaagaaggcgatagaaggcgatgcgctgcgaatcgggagcggcgataccgtaaagcacgaggaagcggtcagcccattcgccgccaagctcttcagcaatatcacgggtagccaacgctatgtcctgatagcggtccgccacacccagccggccacagtcgatgaatccagaaaagcggccattttccaccatgatattcggcaagcaggcatcgccatgggtcacgacgagatcctcgccgtcgggcatccgcgccttgagcctggcgaacagttcggctggcgcgagcccctgatgctcttcgtccagatcatcctgatcgacaagaccggcttccatccgagtacgtgctcgctcgatgcgatgtttcgcttggtggtcgaatgggcaggtagccggatcaagcgtatgcagccgccgcattgcatcagccatgatggatactttctcggcaggagcaaggtgagatgacaggagatcctgccccggcacttcgcccaatagcagccagtcccttcccgcttcagtgacaacgtcgagacagctgcgcaaggaacgcccgtcgtggccagccacgatagccgcgctgcctcgtcttggagttcattcagggcaccggacaggtcggtcttgacaaaaagaaccgggcgcccctgcgctgacagccggaacacggcggcatcagagcagccgattgtctgttgtgcccagtcatagccgaatagcctctccacccaagcggccggagaacctgcgtgcaatccatcttgttcaatcatgcgaaacgatcctcatcctgtctcttgatcagatcttgatcccctgcgccatcagatccttggcggcaagaaagccatccagtttactttgcagggcttcccaaccttaccagagggcgccccagctggcaattccg